European Patent Application EP 4 640 210 A1, published October 29, 2025. Title: Formulations comprising immune stimulating IL-2 analog conjugates. Applicant: HANMI PHARM. CO., LTD. Application KR. The sequence listing filed with the application follows.

SEQUENCE LISTING (130 sequences)

SEQ ID NO: 1 - protein, 133 aa, HOMO SAPIENS [sequence omitted]

SEQ ID NO: 2 - protein, 132 aa, synthetic construct
  REGION 1..132: note = IL-2 analog 1
PTSSSTKKTQLQLEHLLLDLQMILNGINNYKNPKLTRMLTFKFYMPKKATELKHLQCLEEELKPLEEVLNLAQSKNFHLRPRDLISNINVIVLELKGSETTFMCEYADETATIVEFLNRWITFSQSIISTLT

SEQ ID NO: 3 - protein, 132 aa, synthetic construct
  REGION 1..132: note = IL-2 analog 2
PTSSSTKKTQLQLEHLLLDLQMILNGINNYKNPKLTRMLTFKFYMPKKATELKHLQCLEEELKPLEEVLNLAQSKNFHLRPRDLICNINVIVLELKGSETTFMCEYADETATIVEFLNRWITFSQSIISTLT

SEQ ID NO: 4 - protein, 132 aa, synthetic construct
  REGION 1..132: note = IL-2 analog 3
PTSSSTKKTQLQLEHLLLDLQMILNGINNYCNPKLTRMLTFKFYMPKKATELKHLQCLEEELKPLEEVLNLAQSKNFHLRPRDLISNINVIVLELKGSETTFMCEYADETATIVEFLNRWITFSQSIISTLT

SEQ ID NO: 5 - protein, 132 aa, synthetic construct
  REGION 1..132: note = IL-2 analog 4
PTSSSTKKTQLQLEHLLLDLQMILNGINNYKNPCLTRMLTFKFYMPKKATELKHLQCLEEELKPLEEVLNLAQSKNFHLRPRDLISNINVIVLELKGSETTFMCEYADETATIVEFLNRWITFSQSIISTLT

SEQ ID NO: 6 - protein, 132 aa, synthetic construct
  REGION 1..132: note = IL-2 analog 5
PTSSSTKKTQLQLEHLLLDLQMILNGINNYKNPKLTRMLTFCFYMPKKATELKHLQCLEEELKPLEEVLNLAQSKNFHLRPRDLISNINVIVLELKGSETTFMCEYADETATIVEFLNRWITFSQSIISTLT

SEQ ID NO: 7 - protein, 132 aa, synthetic construct
  REGION 1..132: note = IL-2 analog 6
PTSSSTKKTQLQLEHLLLDLQMILNGINNYKNPKLTRMLTFKFYMPCKATELKHLQCLEEELKPLEEVLNLAQSKNFHLRPRDLISNINVIVLELKGSETTFMCEYADETATIVEFLNRWITFSQSIISTLT

SEQ ID NO: 8 - protein, 132 aa, synthetic construct
  REGION 1..132: note = IL-2 analog 7
PTSSSTKKTQLQLEHLLLDLQMILNGINNYKNPKLTRMLTFKFYMPKCATELKHLQCLEEELKPLEEVLNLAQSKNFHLRPRDLISNINVIVLELKGSETTFMCEYADETATIVEFLNRWITFSQSIISTLT

SEQ ID NO: 9 - protein, 132 aa, synthetic construct
  REGION 1..132: note = IL-2 analog 9
PTSSSTKKTQLQLEHLLLDLQMILNGINNYKNPKLTRMLTFKFYMPKKATELKHLQCLEEELKPLEEVLNLAQSCNFHLRPRDLISNINVIVLELKGSETTFMCEYADETATIVEFLNRWITFSQSIISTLT

SEQ ID NO: 10 - protein, 132 aa, synthetic construct
  REGION 1..132: note = IL-2 analog 10
PTSSSTKKTQLQLEHLLLDLQMILNGINNYKNPKLTAMLTFKFYMPKKATELKHLQCLEEELKPLEEVLNLAQSKNFHLRPRDLISNINVIVLELKGSETTFMCEYADETATIVEFLNRWITFSQSIISTLT

SEQ ID NO: 11 - protein, 132 aa, synthetic construct
  REGION 1..132: note = IL-2 analog 10
PTSSSTKKTQLQLEHLLLDLQMILNGINNYKNPKLTRMLTKKFYMPKKATELKHLQCLEEELKPLEEVLNLAQSKNFHLRPRDLISNINVIVLELKGSETTFMCEYADETATIVEFLNRWITFSQSIISTLT

SEQ ID NO: 12 - protein, 132 aa, synthetic construct
  REGION 1..132: note = IL-2 analog 11
PTSSSTKKTQLQLEHLLLDLQMILNGINNYKNPKLTRMLTAKFYMPKKATELKHLQCLEEELKPLEEVLNLAQSKNFHLRPRDLISNINVIVLELKGSETTFMCEYADETATIVEFLNRWITFSQSIISTLT

SEQ ID NO: 13 - protein, 132 aa, synthetic construct
  REGION 1..132: note = IL-2 analog 12
PTSSSTKKTQLQLEHLLLDLQMILNGINNYKNPKLTAMLTKKFYMPKKATELKHLQCLEEELKPLEEVLNLAQSKNFHLRPRDLISNINVIVLELKGSETTFMCEYADETATIVEFLNRWITFSQSIISTLT

SEQ ID NO: 14 - protein, 132 aa, synthetic construct
  REGION 1..132: note = IL-2 analog 13
PTSSSTKKTQLQLEHLLLDLQMILNGINNYKNPKLTAMLTAKFYMPKKATELKHLQCLEEELKPLEEVLNLAQSKNFHLRPRDLISNINVIVLELKGSETTFMCEYADETATIVEFLNRWITFSQSIISTLT

SEQ ID NO: 15 - protein, 132 aa, synthetic construct
  REGION 1..132: note = IL-2 analog 14
PTSSSTKKTQLQLEHLLYDLQMILNGINNYKNPKLTAMLTKKFYMPKKATELKHLQCLEEELKPLEEVLNLAQSKNFHLRPRDLISNINVIVLELKGSETTFMCEYADETATIVEFLNRWITFSQSIISTLT

SEQ ID NO: 16 - protein, 132 aa, synthetic construct
  REGION 1..132: note = IL-2 analog 15
PTSSSTKKTQLQLEHLLLDLQMILNGINNYKNPKLTAMLTKKFYMPKKATELKHLQCLEEELKPLEEVLNLAQSKNFHLRPRELISNINVIVLELKGSETTFMCEYADETATIVEFLNRWITFSQSIISTLT

SEQ ID NO: 17 - protein, 132 aa, synthetic construct
  REGION 1..132: note = IL-2 analog 16
PTSSSTKKTQLQLEHLLLDLQMILNGINNYKNPKLTAMLTKKFYMPKKATELKHLQCLEEELKPLEEVLNLAQSKNFHLRPRDLISQINVIVLELKGSETTFMCEYADETATIVEFLNRWITFSQSIISTLT

SEQ ID NO: 18 - protein, 132 aa, synthetic construct
  REGION 1..132: note = IL-2 analog 17
PTSSSTKKTQLQLEHLLLDLQMILNGINNYKNPKLTAMLTKKFYMPKKATELKHLQCLEEELKPLEEVLNLAQSKNFHLRPRDLISNINTIVLELKGSETTFMCEYADETATIVEFLNRWITFSQSIISTLT

SEQ ID NO: 19 - protein, 132 aa, synthetic construct
  REGION 1..132: note = IL-2 analog 18
PTSSSTKKTQLQLEHLLLDLQMILNGINNYKNPKLTAMLTKKFYMPKKATELKHLQCLEQELKPLEEVLNLAQSKNFHLRPRDLISNINVIVLELKGSETTFMCEYADETATIVEFLNRWITFSQSIISTLT

SEQ ID NO: 20 - protein, 132 aa, synthetic construct
  REGION 1..132: note = IL-2 analog 19
PTSSSTKKTQLQLEHLLLDLQMILNGINNYKNPKLTAMLTKKFYMPKKATELKHLQCLEEELKPLEEVLNLAQSKNFHLDPRDLISNINVFVLELKGSETTFMCEYADETATIVEFLNRWITFSQSIISTLT

SEQ ID NO: 21 - protein, 132 aa, synthetic construct
  REGION 1..132: note = IL-2 analog 20
PTSSSTKKTQLQLEHLLLDLQMILNGINNYKNPKLTAMLTKKFYMPKKATELKHLQCLEEELKPLEEVLNLAQSKNFHLRPRDVVSNINVFVLELKGSETTFMCEYADETATIVEFLNRWITFSQSIISTLT

SEQ ID NO: 22 - protein, 132 aa, synthetic construct
  REGION 1..132: note = IL-2 analog 21
PTSSSTKKTQLQLEHLLLDLQMILNGINNYKNPKLTAMLTKKFYMPKKATELKHLQCLEEELKPLEEVLNLAQSKNFHFDPRDVVSNINVFVLELKGSETTFMCEYADETATIVEFLNRWITFSQSIISTLT

SEQ ID NO: 23 - protein, 132 aa, synthetic construct
  REGION 1..132: note = IL-2 analog 22
PTSSSTKKTQVQLEHLLLDLQMILNGINNYKNPKLTAMLTKKFYMPKKATELKHLQCLEEELKPLEEVLNLAQSKNFHLRPRDLISNINVIVLELKGSETTFMCEYADETATIVEFLNRWITFSQSIISTLT

SEQ ID NO: 24 - protein, 132 aa, synthetic construct
  REGION 1..132: note = IL-2 analog 23
PTSSSTKKTQFQLEHLLLDLQMILNGINNYKNPKLTAMLTKKFYMPKKATELKHLQCLEEELKPLEEVLNLAQSKNFHLRPRDLISNINVIVLELKGSETTFMCEYADETATIVEFLNRWITFSQSIISTLT

SEQ ID NO: 25 - protein, 132 aa, synthetic construct
  REGION 1..132: note = IL-2 analog 24
PTSSSTKKTQLQLEHLLVDLQMILNGINNYKNPKLTAMLTKKFYMPKKATELKHLQCLEEELKPLEEVLNLAQSKNFHLRPRDLISNINVIVLELKGSETTFMCEYADETATIVEFLNRWITFSQSIISTLT

SEQ ID NO: 26 - protein, 132 aa, synthetic construct
  REGION 1..132: note = IL-2 analog 25
PTSSSTKKTQLQLEHLLFDLQMILNGINNYKNPKLTAMLTKKFYMPKKATELKHLQCLEEELKPLEEVLNLAQSKNFHLRPRDLISNINVIVLELKGSETTFMCEYADETATIVEFLNRWITFSQSIISTLT

SEQ ID NO: 27 - protein, 132 aa, synthetic construct
  REGION 1..132: note = IL-2 analog 26
PTSSSTKKTQLQLEHLLLDLQMILNGINNYKNPKLTAMLTKKFYMPKKATELKHLQCLEEELKPLEEVLNLAQSKNFHLRPRDLISNFNVIVLELKGSETTFMCEYADETATIVEFLNRWITFSQSIISTLT

SEQ ID NO: 28 - protein, 132 aa, synthetic construct
  REGION 1..132: note = IL-2 analog 27
PTSSSTKKTQLQLEHLLLDLQMILNGINNYKNPKLTAMLTKKFYMPKKATELKHLQCLEEELKPLEEVLNLAQSKNFHLRPRDLISNINFIVLELKGSETTFMCEYADETATIVEFLNRWITFSQSIISTLT

SEQ ID NO: 29 - protein, 132 aa, synthetic construct
  REGION 1..132: note = IL-2 analog 28
PTSSSTKKTQLQLEHLLLDLQMILNGINNYKNPKLTAMLTKKFYMPKKATELKHLQCLEEELKPLEEVLNLAQSKNFHLRPRDLISNINVIVVELKGSETTFMCEYADETATIVEFLNRWITFSQSIISTLT

SEQ ID NO: 30 - protein, 132 aa, synthetic construct
  REGION 1..132: note = IL-2 analog 29
PTSSSTKKTQLQLEHLLLDLQMILNGINNYKNPKLTAMLTKKFYMPKKATELKHLQCLEEELKPLEEVLNLAQSKNFHLRPRDLISNINVIVLELKGSETTFMCEYADETATIVEFLNRWITFSTSIISTLT

SEQ ID NO: 31 - protein, 132 aa, synthetic construct
  REGION 1..132: note = IL-2 analog 30
PTSSSTKKTQLQLEHLLLDLQMILNGINNYKNPKLTAMLTFKFYMPKKATELKHLQCLEEELKPLEEVLNLAQSKNFHLDPRDLISNINVFVLELKGSETTFMCEYADETATIVEFLNRWITFSQSIISTLT

SEQ ID NO: 32 - protein, 132 aa, synthetic construct
  REGION 1..132: note = IL-2 analog 31
PTSSSTKKTQLQLEHLLLDLQMILNGINNYKNPKLTAMLTFKFYMPKKATELKHLQCLEEELKPLEEVLNLAQSKNFHLRPRELISNINVIVLELKGSETTFMCEYADETATIVEFLNRWITFSQSIISTLT

SEQ ID NO: 33 - protein, 132 aa, synthetic construct
  REGION 1..132: note = IL-2 analog 32
PTSSSTKKTQLQLEHLLLDLQMILNGINNYKNPKLTAMLTFKFYMPKKATELKHLQCLEEELKPLEEVLNLAQSKNFHLDPRELISNINVFVLELKGSETTFMCEYADETATIVEFLNRWITFSQSIISTLT

SEQ ID NO: 34 - protein, 132 aa, synthetic construct
  REGION 1..132: note = IL-2 analog 33
PTSSSTKKTQLQLEHLLLDLQMILNGINNYKNPKLTAMLTFKFYMPKKATELKHLQCLEEELKPLEEVLNLAQSKNFHFRPRDLISNINVIVLELKGSETTFMCEYADETATIVEFLNRWITFSQSIISTLT

SEQ ID NO: 35 - protein, 132 aa, synthetic construct
  REGION 1..132: note = IL-2 analog 34
PTSSSTKKTQLQLEHLLLDLQMILNGINNYKNPKLTAMLTFKFYMPKKATELKHLQCLEEELKPLEEVLNLAQSKNFHFRPRELISNINVIVLELKGSETTFMCEYADETATIVEFLNRWITFSQSIISTLT

SEQ ID NO: 36 - protein, 132 aa, synthetic construct
  REGION 1..132: note = IL-2 analog 35
PTSSSTKKTQLQLEHLLLDLQMILNGINNYKNPKLTAMLTFKFYMPKKATELKHLQCLEEELKPLEEVLNLAQSKNFHLRPRDLISNINVIVFEFKGSETTFMCEYADETATIVEFLNRWITFSQSIISTLT

SEQ ID NO: 37 - protein, 132 aa, synthetic construct
  REGION 1..132: note = IL-2 analog 36
PTSSSTKKTQLQLEHLLLDLQMILNGINNYKNPKLTAMLTFKFYMPKKATELKHLQCLEEELKPLEEVLNLAQSKNFHLRPRDLISNINVIVFEVKGSETTFMCEYADETATIVEFLNRWITFSQSIISTLT

SEQ ID NO: 38 - protein, 132 aa, synthetic construct
  REGION 1..132: note = IL-2 analog 37
PTSSSTKKTQLQLEHLLLDLQMILNGINNYKNPKLTAMLTFKFYMPKKATELKHLQCLEEELKPLEEVLNLAQSKNFHLRPRDLISNINVIVFEIKGSETTFMCEYADETATIVEFLNRWITFSQSIISTLT

SEQ ID NO: 39 - protein, 132 aa, synthetic construct
  REGION 1..132: note = IL-2 analog 38
PTSSSTKKTQLQLEHLLLDLQMILNGINNYKNPKLTAMLTKKFYMPKKATELKHLQCLEEELKPLEEVLNLAQSKNFHLDPRDLISNINVFVFEFKGSETTFMCEYADETATIVEFLNRWITFSQSIISTLT

SEQ ID NO: 40 - protein, 132 aa, synthetic construct
  REGION 1..132: note = IL-2 analog 39
PTSSSTKKTQLQLEHLLLDLQMILNGINNYKNPKLTAMLTKKFYMPKKATELKHLQCLEEELKPLEEVLNLAQSKNFHLDPRDLISNINVFVFEVKGSETTFMCEYADETATIVEFLNRWITFSQSIISTLT

SEQ ID NO: 41 - protein, 132 aa, synthetic construct
  REGION 1..132: note = IL-2 analog 40
PTSSSTKKTQLQLEHLLLDLQMILNGINNYKNPKLTAMLTKKFYMPKKATELKHLQCLEEELKPLEEVLNLAQSKNFHLDPRDLISNINVFVFEIKGSETTFMCEYADETATIVEFLNRWITFSQSIISTLT

SEQ ID NO: 42 - protein, 132 aa, synthetic construct
  REGION 1..132: note = IL-2 analog 41
PTSSSTKKTQLQLEHLLLDLQMILNGINNYKNPKLTRMLTFKFYMPKKATELKHLQCLEEELKPLEEVLNLAQSKNFHFDPRDVVSNINVFVLELKGSETTFMCEYADETATIVEFLNRWITFSQSIISTLT

SEQ ID NO: 43 - protein, 132 aa, synthetic construct
  REGION 1..132: note = IL-2 analog 42
PTSSSTKKTQLQLEHLLLDLQMILNGINNYKNPKLTAMLTKKFYMPKKATELKHLQCLEEELKPLEEVLNLAQSKNFHLEPRDLISNINVFVLELKGSETTFMCEYADETATIVEFLNRWITFSQSIISTLT

SEQ ID NO: 44 - protein, 132 aa, synthetic construct
  REGION 1..132: note = IL-2 analog 43
PTSSSTKKTQLQLEHLLLDLQMILNGINNYKNPKLTAMLTKKFYMPKKATELKHLQCLEEELKPLEEVLNLAQSKNFHLDPRDLISNINVLVLELKGSETTFMCEYADETATIVEFLNRWITFSQSIISTLT

SEQ ID NO: 45 - protein, 132 aa, synthetic construct
  REGION 1..132: note = IL-2 analog 44
PTSSSTKKTQLQLEHLLLDLQMILNGINNYKNPKLTAMLTKKFYMPKKATELKHLQCLEEELKPLEEVLNLAQSKNFHLDPRVLISNINVFVLELKGSETTFMCEYADETATIVEFLNRWITFSQSIISTLT

SEQ ID NO: 46 - protein, 132 aa, synthetic construct
  REGION 1..132: note = IL-2 analog 45
PTSSSTKKTQLQLEHLLLDLQMILNGINNYKNPKLTAMLTKKFYMPKKATELKHLQCLEEELKPLEEVLNLAQSKNFHLDPRFLISNINVFVLELKGSETTFMCEYADETATIVEFLNRWITFSQSIISTLT

SEQ ID NO: 47 - protein, 132 aa, synthetic construct
  REGION 1..132: note = IL-2 analog 46
PTSSSTKKTQLQLEHLLLVLQMILNGINNYKNPKLTAMLTKKFYMPKKATELKHLQCLEEELKPLEEVLNLAQSKNFHLDPRDLISNINVFVLELKGSETTFMCEYADETATIVEFLNRWITFSQSIISTLT

SEQ ID NO: 48 - protein, 132 aa, synthetic construct
  REGION 1..132: note = IL-2 analog 47
PTSSSTKKTQLQLEHLLLFLQMILNGINNYKNPKLTAMLTKKFYMPKKATELKHLQCLEEELKPLEEVLNLAQSKNFHLDPRDLISNINVFVLELKGSETTFMCEYADETATIVEFLNRWITFSQSIISTLT

SEQ ID NO: 49 - protein, 132 aa, synthetic construct
  REGION 1..132: note = IL-2 analog 48
PTSSSTKKTQLQLEHLLLDLQMILNGINNYKNPKLTAMLTKKFYMPKKATELKHLQCLEEELKPLEEVLNLAQSKNFHLDPRDLISVINVFVLELKGSETTFMCEYADETATIVEFLNRWITFSQSIISTLT

SEQ ID NO: 50 - protein, 132 aa, synthetic construct
  REGION 1..132: note = IL-2 analog 49
PTSSSTKKTQLQLEHLLLDLQMILNGINNYKNPKLTAMLTKKFYMPKKATELKHLQCLEEELKPLEEVLNLAQSKNFHLDPRDLISFINVFVLELKGSETTFMCEYADETATIVEFLNRWITFSQSIISTLT

SEQ ID NO: 51 - protein, 132 aa, synthetic construct
  REGION 1..132: note = IL-2 analog 50
PTSSSTKKTQLQLEHLLLDLQMILNGINNYKNPKLTRMLTKKFYMPKKATELKHLQCLEEELKPLEEVLNLAQSKNFHFDPRDVVSNINVFVLELKGSETTFMCEYADETATIVEFLNRWITFSQSIISTLT

SEQ ID NO: 52 - protein, 132 aa, synthetic construct
  REGION 1..132: note = IL-2 analog 51
PTSSSTKKTQLQLEHLLLDLQMILNGINNYKNPKLTRMLTFKFYMPKKATELKHLQCLEQELKPLEEVLNLAQSKNFHLDPRDLISNINVFVLELKGSETTFMCEYADETATIVEFLNRWITFSQSIISTLT

SEQ ID NO: 53 - protein, 132 aa, synthetic construct
  REGION 1..132: note = IL-2 analog 52
PTSSSTKKTQLQLEHLLLDLQMILNGINNYKNPKLTAMLTKKFYMPKKATELKHLQCLEEELKPLEEVLNLAQSKNFHFDPRDLISNINVFVLELKGSETTFMCEYADETATIVEFLNRWITFSQSIISTLT

SEQ ID NO: 54 - protein, 132 aa, synthetic construct
  REGION 1..132: note = IL-2 analog 53
PTSSSTKKTQLQLEHLLLDLQMILNGINNYKNPKLTAMLTKKFYMPKKATELKHLQCLEEELKPLEEVLNLAQSKNFHFDPRELISNINVFVLELKGSETTFMCEYADETATIVEFLNRWITFSQSIISTLT

SEQ ID NO: 55 - protein, 132 aa, synthetic construct
  REGION 1..132: note = IL-2 analog 54
PTSSSTKKTQLQLEHLLLDLQMILNGINNYKNPKLTAMLTKKFYMPKKATELKHLQCLEEELKPLEEVLNLAHSKNFHLDPRDLISNINVFVLELKGSETTFMCEYADETATIVEFLNRWITFSQSIISTLT

SEQ ID NO: 56 - protein, 132 aa, synthetic construct
  REGION 1..132: note = IL-2 analog 55
PTSSSTKKTQLQLEHLLLDLQMILNGINNYKNPKLTAMLTKKFYMPKKATELKHLQCLEEELKPLEEVLNLAHSKNFHFDPRDLISNINVFVLELKGSETTFMCEYADETATIVEFLNRWITFSQSIISTLT

SEQ ID NO: 57 - protein, 132 aa, synthetic construct
  REGION 1..132: note = IL-2 analog 56
PTSSSTKKTQLQLEHLLLDLQMILNGINNYKNPKLTAMLTKKFAMPKKATELKHLQCLEEELKPLEEVLNLAHSKNFHLDPRDLISNINVFVLELKGSETTFMCEYADETATIVEFLNRWITFSQSIISTLT

SEQ ID NO: 58 - protein, 132 aa, synthetic construct
  REGION 1..132: note = IL-2 analog 57
PTSSSTKKTQLQLEHLLLDLQMILNGINNYKNPKLTAMLTKKFAMPKKATELKHLQCLEEELKPLEEVLNLAHSKNFHFDPRDLISNINVFVLELKGSETTFMCEYADETATIVEFLNRWITFSQSIISTLT

SEQ ID NO: 59 - protein, 132 aa, synthetic construct
  REGION 1..132: note = IL-2 analog 61
PTSSSTKKTQLQLEHLLLDLQMILNGINNYKNPKLTAMLTKKFYMPKKATELKHLQCLEEELKPLEEVLNLAQSKNFHFDPRDAASNINVFVLELKGSETTFMCEYADETATIVEFLNRWITFSQSIISTLT

SEQ ID NO: 60 - protein, 132 aa, synthetic construct
  REGION 1..132: note = IL-2 analog 59
PTSSSTKKTQLQLEHLLLDLQMILNGINNYKNPKLTAMLTKKFYMPKKATELKHLQCLEEELKPLEEVLNLAQSKNFHFDPRDAASNINVYVLELKGSETTFMCEYADETATIVEFLNRWITFSQSIISTLT

SEQ ID NO: 61 - protein, 132 aa, synthetic construct
  REGION 1..132: note = IL-2 analog 60
PTSSSTKKTQLQLEHLLLDLQMILNGINNYKNPKLTAMLTKKFAMPKKATELKHLQCLEEELKPLEEVLNLAQSKNFHYRPRDAASNINVYVLELKGSETTFMCEYADETATIVEFLNRWITFSQSIISTLT

SEQ ID NO: 62 - protein, 132 aa, synthetic construct
  REGION 1..132: note = IL-2 analog 61
PTSSSTKKTQLQLEHLLLDLQMILNGINNYKNPKLTAMLTKKFYMPKKATELKHLQCLEEELKPLEEVLNLAQSKNFHYDPRDGVSNINVYVLELKGSETTFMCEYADETATIVEFLNRWITFSQSIISTLT

SEQ ID NO: 63 - protein, 132 aa, synthetic construct
  REGION 1..132: note = IL-2 analog 62
PTSSSTKKTQLQLEHLLLDLQMILNGINNYKNPKLTAMLTKKFYMPKKATELKHLQCLEEELKPLEEVLNLAQSKNFHWEPRDGASNINVFVLELKGSETTFMCEYADETATIVEFLNRWITFSQSIISTLT

SEQ ID NO: 64 - protein, 132 aa, synthetic construct
  REGION 1..132: note = IL-2 analog 63
PTSSSTKKTQLQLEHLLLDLQMILNGINNYKNPKLTAMLTKKFYMPKKATELKHLQCLEEELKPLEEVLNLAQSKNFHDEPRDTGSNINVFVLELKGSETTFMCEYADETATIVEFLNRWITFSQSIISTLT

SEQ ID NO: 65 - protein, 132 aa, synthetic construct
  REGION 1..132: note = IL-2 analog 64
PTSSSTKKTQLQLEHLLLDLQMILNGINNYKNPKLTAMLTKKFYMPKKATELKHLQCLEEELKPLEEVLNLAQSKNFHYNPRDVVSNINVYVLELKGSETTFMCEYADETATIVEFLNRWITFSQSIISTLT

SEQ ID NO: 66 - protein, 132 aa, synthetic construct
  REGION 1..132: note = IL-2 analog 65
PTSSSTKKTQLQLEHLLLDLQMILNGINNYKNPKLTAMLTKKFYMPKKATELKHLQCLEEELKPLEEVLNLAQSKNFHYEPRDVVSNINVFVLELKGSETTFMCEYADETATIVEFLNRWITFSQSIISTLT

SEQ ID NO: 67 - protein, 132 aa, synthetic construct
  REGION 1..132: note = IL-2 analog 66
PTSSSTKKTQLQLEHLLLDLQMILNGINNYKNPKLTAMLTKKFYMPKKATELKHLQCLEEELKPLEEVLNLAQSKNFHFEPRDFVSNINVFVLELKGSETTFMCEYADETATIVEFLNRWITFSQSIISTLT

SEQ ID NO: 68 - protein, 132 aa, synthetic construct
  REGION 1..132: note = IL-2 analog 67
PTSSSTKKTQLQLEHLLLDLQMILNGINNYKNPKLTAMLTKKFYMPKKATELKHLQCLEEELKPLEEVLNLAQSKNFHYDPRDFVSNINVWVLDLKGSETTFMCEYADETATIVEFLNRWITFSQSIISTLT

SEQ ID NO: 69 - protein, 132 aa, synthetic construct
  REGION 1..132: note = IL-2 analog 68
PTSSSTKKTQLQLEHLLLDLQMILNGINNYKNPKLTAMLTKKFYMPKKATELKHLQCLEEELKPLEEVLNLAQSKNFHFEPRDIVSNINEFVLELKGSETTFMCEYADETATIVEFLNRWITFSQSIISTLT

SEQ ID NO: 70 - protein, 132 aa, synthetic construct
  REGION 1..132: note = IL-2 analog 69
PTSSSTKKTQLQLEHLLLDLQMILNGINNYKNPKLTAMLTKKFYMPKKATELKHLQCLEEELKPLEEVLNLAQSKNFHYEPRDFLSNINEWVLDLKGSETTFMCEYADETATIVEFLNRWITFSQSIISTLT

SEQ ID NO: 71 - protein, 132 aa, synthetic construct
  REGION 1..132: note = IL-2 analog 70
PTSSSTKKTQLQLEHLLLDLQMILNGINNYKNPKLTAMLTKKFYMPKKATELKHLQCLEEELKPLEEVLNLAQSKNFHYDPRDVVSNINVFVLELKGSETTFMCEYADETATIVEFLNRWITFSQSIISTLT

SEQ ID NO: 72 - protein, 132 aa, synthetic construct
  REGION 1..132: note = IL-2 analog 71
PTSSSTKKTQLQLEHLLLDLQMILNGINNYKNPKLTAMLTKKFYMPKKATELKHLQCLEEELKPLEEVLNLAQSKNFHFEPRDVVSNINVFVLELKGSETTFMCEYADETATIVEFLNRWITFSQSIISTLT

SEQ ID NO: 73 - protein, 132 aa, synthetic construct
  REGION 1..132: note = IL-2 analog 72
PTSSSTKKTQLQLEHLLLDLQMILNGINNYKNPKLTAMLTKKFYMPKKATELKHLQCLEEELKPLEEVLNLAQSKNFHFDPRDVGSNINVFVLELKGSETTFMCEYADETATIVEFLNRWITFSQSIISTLT

SEQ ID NO: 74 - protein, 132 aa, synthetic construct
  REGION 1..132: note = IL-2 analog 73
PTSSSTKKTQLQLEHLLLDLQMILNGINNYKNPKLTAMLTKKFYMPKKATELKHLQCLEEELKPLEEVLNLAQSKNFHFDPRDWVSNINVFVLELKGSETTFMCEYADETATIVEFLNRWITFSQSIISTLT

SEQ ID NO: 75 - protein, 132 aa, synthetic construct
  REGION 1..132: note = IL-2 analog 74
PTSSSTKKTQLQLEHLLLDLQMILNGINNYKNPKLTDMLTKKFYMPKKATELKHLQCLEEELKPLEEVLNLAQSKNFHYDPRDVVSNINVFVLELKGSETTFMCEYADETATIVEFLNRWITFSQSIISTLT

SEQ ID NO: 76 - protein, 132 aa, synthetic construct
  REGION 1..132: note = IL-2 analog 75
PTSSSTKKTQLQLEHLLLDLQMILNGINNYKNPKLTAMLTKKFAMPKKATELKHLQCLEEELKPLEEVLNLAQSKNFHFEPRDVVSNINVFVLELKGSETTFMCEYADETATIVEFLNRWITFSQSIISTLT

SEQ ID NO: 77 - protein, 132 aa, synthetic construct
  REGION 1..132: note = IL-2 analog 76
PTSSSTKKTQLQLEHLLLDLQMILNGINNYKNPKLTAMLTKQFYMPKKATELKHLQCLERELKPLEEVLNLAQSKNFHFDPRDVGSNINVFVLELKGSETTFMCEYADETATIVEFLNRWITFSQSIISTLT

SEQ ID NO: 78 - protein, 132 aa, synthetic construct
  REGION 1..132: note = IL-2 analog 77
PTSSSTKKTQLQLEHLLLDLQMILNGINNYKNPKLTAMLTKEFYMPKKATELKHLQCLERELKPLEEVLNLAQSKNFHFDPRDWVSNINVFVLELKGSETTFMCEYADETATIVEFLNRWITFSQSIISTLT

SEQ ID NO: 79 - protein, 132 aa, synthetic construct
  REGION 1..132: note = IL-2 analog 78
PTSSSTKKTQLQLEHLLLDLQMILNGINNYKNPELTAMLTKKFYMPKKATELKHLQCLEEELKPLEEVLNLAQSKNFHFEPRDVVSNINVFVLELKGSETTFMCEYADETATIVEFLNRWITFSQSIISTLT

SEQ ID NO: 80 - protein, 132 aa, synthetic construct
  REGION 1..132: note = IL-2 analog 79
PTSSSTKKTQLQLEHLLLDLQMILNGINNYKNPELTAMLTKKFYMPKKATELKHLQCLEEELKPLEEVLNLAHSKNFHFEPRDVVSNINVFVLELKGSETTFMCEYADETATIVEFLNRWITFSQSIISTLT

SEQ ID NO: 81 - protein, 132 aa, synthetic construct
  REGION 1..132: note = IL-2 analog 80
PTSSSTKKTQLQLEHLLLDLQMILNGINNYKNPELTAMLTKKFYMPKKATELKHLQCLEEELKPLEEVLNLAHSKNFHFEGRDVVSNINVFVLELKGSETTFMCEYADETATIVEFLNRWITFSQSIISTLT

SEQ ID NO: 82 - protein, 132 aa, synthetic construct
  REGION 1..132: note = IL-2 analog 81
PTSSSTKKTQLQLEHLLLDLQMILNGINNYKNPELTAMLTKKFYMPKKATELKHLQCLEEELKPLEEVLNLAHSKNFHFEVRDVVSNINVFVLELKGSETTFMCEYADETATIVEFLNRWITFSQSIISTLT

SEQ ID NO: 83 - protein, 132 aa, synthetic construct
  REGION 1..132: note = IL-2 analog 82
PTSSSTKKTQLQLEHLRLDLEMILNGINNYKNPKLTRMLTFKFYMPKKATELKHLQCLEEELKPLEEVLNLAQSKNFHFDPRDEVSNINVFVLELKGSETTFMCEYADETATIVEFLNRWITFSQSIISTLT

SEQ ID NO: 84 - protein, 132 aa, synthetic construct
  REGION 1..132: note = IL-2 analog 83
PTSSSTKKTQLQLEHLRRDLEMILNGINNYKNPKLTRMLTFKFYMPKKATELKHLQCLEEELKPLEEVLNLAQSKNFHFDPRDEVSNINVFVLELKGSETTFMCEYADETATIVEFLNRWITFSQSIISTLT

SEQ ID NO: 85 - protein, 132 aa, synthetic construct
  REGION 1..132: note = IL-2 analog 84
PTSSSTKKTQLQLEHLRLDLEMILNGINNYKNPKLTRMLTFKFYMPKKATELKHLQCLEEELKPLEEVLNLAQSKNFHVDPRDEVSNINVFVLELKGSETTFMCEYADETATIVEFLNRWITFSQSIISTLT

SEQ ID NO: 86 - protein, 132 aa, synthetic construct
  REGION 1..132: note = IL-2 analog 85
PTSSSTKKTQLQLEHLLLDLQMILNGINNYKNPKLTRMLTFKFYMPKKATELKHLQCLEEELKPLEEVLNLAQSKNFHFEPRDVVSNINVFVLELKGSETTFMCEYADETATIVEFLNRWITFSQSIISTLT

SEQ ID NO: 87 - protein, 132 aa, synthetic construct
  REGION 1..132: note = IL-2 analog 86
PTSSSTKKTQLQLEHLRLDLEMILNGINNYKNPKLTRMLTFKFYMPKKATELKHLQCLEEELKPLEEVLNLAQSKNFHFEPRDVVSNINVFVLELKGSETTFMCEYADETATIVEFLNRWITFSQSIISTLT

SEQ ID NO: 88 - protein, 132 aa, synthetic construct
  REGION 1..132: note = IL-2 analog 87
PTSSSTKKTQLQLEHLRRDLEMILNGINNYKNPKLTRMLTFKFYMPKKATELKHLQCLEEELKPLEEVLNLAQSKNFHFEPRDVVSNINVFVLELKGSETTFMCEYADETATIVEFLNRWITFSQSIISTLT

SEQ ID NO: 89 - protein, 132 aa, synthetic construct
  REGION 1..132: note = IL-2 analog 88
PTSSSTKKTQLQLEHLLLDLQMILNGINNYKNPKLTRMLTFKFYMPKKATELKHLQCLEDELKPLEEVLNLAQSKNFHFEPRDVVSNINVFVLELKGSETTFMCEYADETATIVEFLNRWITFSQSIISTLT

SEQ ID NO: 90 - protein, 132 aa, synthetic construct
  REGION 1..132: note = IL-2 analog 89
PTSSSTKKTQLQLEHLLLDLQMILNGINNYKNPKLTAMLTFKFYMPKKATELKHLQCLEEELKPLEQVLNLAQSKNFHFEPRDVVSNINVFVLELKGSETTFMCEYADETATIVEFLNRWITFSQSIISTLT

SEQ ID NO: 91 - protein, 132 aa, synthetic construct
  REGION 1..132: note = IL-2 analog 90
PTSSSTKKTQLQLEHLLLDLQMILNGINNYKNPKLTRMLTWKFYMPKKATELKHLQCLEEELKPLEEVLNLAQSKNFHFEPRDVVSNINVFVLELKGSETTFMCEYADETATIVEFLNRWITFSQSIISTLT

SEQ ID NO: 92 - protein, 132 aa, synthetic construct
  REGION 1..132: note = IL-2 analog 91
PTSSSTKKTQLQLEHLLLDLQMILNGINNYKNPKLTRMLTFKFYMPKKATELKHLQCLEQELKPLEEVLNLAQSKNFHFEPRDVVSNINVFVLELKGSETTFMCEYADETATIVEFLNRWITFSQSIISTLT

SEQ ID NO: 93 - protein, 132 aa, synthetic construct
  REGION 1..132: note = IL-2 analog 92
PTSSSTKKTQLQLEHLLLDLQMILNGINNYKNPKLTRMLTFKFYMPKKATELKHLQCLEEELKPLEEVLNLAQSKNFHFEPRDVVSNINTFVLELKGSETTFMCEYADETATIVEFLNRWITFSQSIISTLT

SEQ ID NO: 94 - protein, 132 aa, synthetic construct
  REGION 1..132: note = IL-2 analog 93
PTSSSTKKTQLQLEHLLLDLQMILNGINNYKNPKLTRMLTFKFYMPKKATELKHLQCLEEELKPLEEVLNLAQSKNFHFEPREVVSNINTFVLELKGSETTFMCEYADETATIVEFLNRWITFSQSIISTLT

SEQ ID NO: 95 - protein, 132 aa, synthetic construct
  REGION 1..132: note = IL-2 analog 94
PTSSSTKKTQLQLEHLLLDLQMILNGINNYKNPKLTRMLTFKFYMPKKATELKHLQCLEEELKPLEEVLNLAQSKNFHFEPRDVVSNINVFVFEFKGSETTFMCEYADETATIVEFLNRWITFSQSIISTLT

SEQ ID NO: 96 - protein, 132 aa, synthetic construct
  REGION 1..132: note = IL-2 analog 95
PTSSSTKKTQLQLEHLLLDLQMILNGINNYKNPKLTRMLTFKFYMPKKATELKHLQCLEEELKPLEEGLNLAQSKNFHFEPRDVVSNINVFVLELKGSETTFMCEYADETATIVEFLNRWITFSQSIISTLT

SEQ ID NO: 97 - protein, 132 aa, synthetic construct
  REGION 1..132: note = IL-2 analog 96
PTSSSTKKTQLQLEHLLLDLQMILNGINNYKNPKLTRMLTFKFYMPKKATELKHLQCLEEELKPLEEGLNLAASKNFHFEPRDVVSNINVFVLELKGSETTFMCEYADETATIVEFLNRWITFSQSIISTLT

SEQ ID NO: 98 - protein, 132 aa, synthetic construct
  REGION 1..132: note = IL-2 analog 97
PTSSSTKKTQLQLEHLLLDLQMILNGINNYKNPKLTAMLTFKFYMPKKATELKHLQCLEEELKPLEEVLNLAQSKNFHFDPRDLISNINVFVLELKGSETTFMCEYADETATIVEFLNRWITFSQSIISTLT

SEQ ID NO: 99 - protein, 132 aa, synthetic construct
  REGION 1..132: note = IL-2 analog 98
PTSSSTKKTQLQLEHLLLDLQMILNGINNYKNPKLTAMLTFKFYMPKKATELKHLQCLEEELKPLEEVLNLAQSKNFHFEPRDVISNINVFVLELKGSETTFMCEYADETATIVEFLNRWITFSQSIISTLT

SEQ ID NO: 100 - protein, 132 aa, synthetic construct
  REGION 1..132: note = IL-2 analog 99
PTSSSTKKTQLQLEHLLLDLQMILNGINNYKNPKLTAMLTFKFYMPKKATELKHLQCLEEELKPLEEVLNLAQSKNFHFEPRDLVSNINVFVLELKGSETTFMCEYADETATIVEFLNRWITFSQSIISTLT

SEQ ID NO: 101 - protein, 132 aa, synthetic construct
  REGION 1..132: note = IL-2 analog 100
PTSSSTKKTQLQLEHLLLDLQMILNGINNYKNPKLTRMLTFKFYMPKKATELKHLQCLEEELKPLEEVLNLAQSKNFHFEPRDYVSNINVFVLELKGSETTFMCEYADETATIVEFLNRWITFSQSIISTLT

SEQ ID NO: 102 - protein, 132 aa, synthetic construct
  REGION 1..132: note = IL-2 analog 101
PTSSSTKKTQLQLEHLLLDLQMILNGINNYKNPKLTRMLTFKFYMPKKATELKHLQCLEEELKPLEEVLNLAQSKNFHFEPRDLASNINVFVLELKGSETTFMCEYADETATIVEFLNRWITFSQSIISTLT

SEQ ID NO: 103 - protein, 132 aa, synthetic construct
  REGION 1..132: note = IL-2 analog 102
PTSSSTKKTQLQLEHLLLDLQMILNGINNYKNPKLTRMLTFKFYMPKKATELKHLQCLEEELKPLEEVLNLAQSKNFHFEPRDVVSNINVIVLELKGSETTFMCEYADETATIVEFLNRWITFSQSIISTLT

SEQ ID NO: 104 - protein, 132 aa, synthetic construct
  REGION 1..132: note = IL-2 analog 103
PTSSSTKKTQLQLEHLRLDLEMILNGINNYKNPKLTAMLTFKFYMPKKATELKHLQCLEEELKPLEEVLNLAQSKNFHFEPRDVVSNINVFVLELKGSETTFMCEYADETATIVEFLNRWITFSQSIISTLT

SEQ ID NO: 105 - protein, 132 aa, synthetic construct
  REGION 1..132: note = IL-2 analog 104
PTSSSTKKTQLQLEHLRLDLEMILNGINNYKNPKLTRMLTFKFYMPKKATELKHLQCLEDELKPLEEVLNLAQSKNFHFEPRDVVSNINVFVLELKGSETTFMCEYADETATIVEFLNRWITFSQSIISTLT

SEQ ID NO: 106 - protein, 132 aa, synthetic construct
  REGION 1..132: note = IL-2 analog 105
PTSSSTKKTQLQLEHLRLDLEMILNGINNYKNPKLTRMLTFKFYMPKKATELKHLQCLEEELKPLEDVLNLAQSKNFHFEPRDVVSNINVFVLELKGSETTFMCEYADETATIVEFLNRWITFSQSIISTLT

SEQ ID NO: 107 - protein, 12 aa, HOMO SAPIENS
ESKYGPPCPSCP

SEQ ID NO: 108 - protein, 11 aa, synthetic construct
  REGION 1..11: note = Variant of hinge region
ESKYGPPPSCP

SEQ ID NO: 109 - protein, 11 aa, synthetic construct
  REGION 1..11: note = Variant of hinge region
ESKYGPPCPSP

SEQ ID NO: 110 - protein, 10 aa, synthetic construct
  REGION 1..10: note = Variant of hinge region
ESKYGPPCPS

SEQ ID NO: 111 - protein, 10 aa, synthetic construct
  REGION 1..10: note = Variant of hinge region
ESKYGPPCPP

SEQ ID NO: 112 - protein, 8 aa, synthetic construct
  REGION 1..8: note = Variant of hinge region
KYGPPCPS

SEQ ID NO: 113 - protein, 8 aa, synthetic construct
  REGION 1..8: note = Variant of hinge region
ESKYGPPC

SEQ ID NO: 114 - protein, 7 aa, synthetic construct
  REGION 1..7: note = Variant of hinge region
EKYGPPC

SEQ ID NO: 115 - protein, 6 aa, synthetic construct
  REGION 1..6: note = Variant of hinge region
ESPSCP

SEQ ID NO: 116 - protein, 5 aa, synthetic construct
  REGION 1..5: note = Variant of hinge region
EPSCP

SEQ ID NO: 117 - protein, 4 aa, synthetic construct
  REGION 1..4: note = Variant of hinge region
PSCP

SEQ ID NO: 118 - protein, 10 aa, synthetic construct
  REGION 1..10: note = Variant of hinge region
ESKYGPPSCP

SEQ ID NO: 119 - protein, 9 aa, synthetic construct
  REGION 1..9: note = Variant of hinge region
KYGPPPSCP

SEQ ID NO: 120 - protein, 9 aa, synthetic construct
  REGION 1..9: note = Variant of hinge region
ESKYGPSCP

SEQ ID NO: 121 - protein, 8 aa, synthetic construct
  REGION 1..8: note = Variant of hinge region
ESKYGPPC

SEQ ID NO: 122 - protein, 7 aa, synthetic construct
  REGION 1..7: note = Variant of hinge region
KYGPPCP

SEQ ID NO: 123 - protein, 7 aa, synthetic construct
  REGION 1..7: note = Variant of hinge region
ESKPSCP

SEQ ID NO: 124 - protein, 6 aa, synthetic construct
  REGION 1..6: note = Variant of hinge region
ESPSCP

SEQ ID NO: 125 - protein, 4 aa, synthetic construct
  REGION 1..4: note = Variant of hinge region
EPSC

SEQ ID NO: 126 - skipped

SEQ ID NO: 127 - protein, 133 aa, synthetic construct
  REGION 1..133: note = General Formula 1
  SITE 1: note = X is absent
  SITE 18: note = X is leucine (L) or arginine (R)
  SITE 19: note = X is leucine (L) or tyrosine (Y)
  SITE 22: note = X is glutamic acid (E) or glutamine (Q)
  SITE 38: note = X is alanine (A), aspartic acid (D), or arginine (R)
  SITE 42: note = X is alanine (A), phenylalanine (F), lysine (K), or tryptophan (W)
  SITE 43: note = X is glutamic acid (E), lysine (K), or glutamine (Q)
  SITE 45: note = X is alanine (A) or tyrosine (Y)
  SITE 61: note = X is aspartic acid (D), glutamic acid (E), glutamine (Q), or arginine (R)
  SITE 68: note = X is aspartic acid (D) or glutamic acid (E)
  SITE 74: note = X is histidine (H) or glutamine (Q)
  SITE 80: note = X is phenylalanine (F), leucine (L), valine (V), or tyrosine (Y)
  SITE 81: note = X is aspartic acid (D), glutamic acid (E), or arginine (R)
  SITE 84: note = X is aspartic acid (D) or glutamic acid (E)
  SITE 85: note = X is alanine (A), glutamic acid (E), glycine (G), leucine (L), valine (V), tryptophan (W), or tyrosine (Y)
  SITE 86: note = X is alanine (A), glycine (G), isoleucine (I), or valine (V)
  SITE 91: note = X is threonine (T) or valine (V)
  SITE 92: note = X is phenylalanine (F), isoleucine (I), or tyrosine (Y)
  SITE 94: note = X is phenylalanine (F) or leucine (L)
  SITE 96: note = X is phenylalanine (F) or leucine (L)
XPTSSSTKKTQLQLEHLXXDLXMILNGINNYKNPKLTXMLTXXFXMPKKATELKHLQCLEXELKPLEXVLNLAXSKNFHXXPRXXXSNINXXVXEXKGSETTFMCEYADETATIVEFLNRWITFSQSIISTLT

SEQ ID NO: 128 - protein, 133 aa, synthetic construct
  REGION 1..133: note = General Formula 2
  SITE 1: note = X is absent
  SITE 18: note = X is leucine (L) or arginine (R)
  SITE 22: note = X is glutamic acid (E) or glutamine (Q)
  SITE 38: note = X is alanine (A) or arginine (R)
  SITE 42: note = X is phenylalanine (F) or lysine (K)
  SITE 61: note = X is aspartic acid (D) or glutamic acid (E)
  SITE 68: note = X is aspartic acid (D) or glutamic acid (E)
  SITE 81: note = X is aspartic acid (D) or glutamic acid (E)
  SITE 85: note = X is leucine (L) or valine (V)
  SITE 86: note = X is isoleucine (I) or valine (V)
XPTSSSTKKTQLQLEHLXLDLXMILNGINNYKNPKLTXMLTXKFYMPKKATELKHLQCLEXELKPLEXVLNLAQSKNFHFXPRDXXSNINVFVLELKGSETTFMCEYADETATIVEFLNRWITFSQSIISTLT

SEQ ID NO: 129 - protein, 221 aa, HOMO SAPIENS
PSCPAPEFLGGPSVFLFPPKPKDTLMISRTPEVTCVVVDVSQEDPEVQFNWYVDGVEVHNAKTKPREEQFNSTYRVVSVLTVLHQDWLNGKEYKCKVSNKGLPSSIEKTISKAKGQPREPQVYTLPPSQEEMTKNQVSLTCLVKGFYPSDIAVEWESNGQPENNYKTTPPVLDSDGSFFLYSRLTVDKSRWQEGNVFSCSVMHEALHNHYTQKSLSLSLGK

SEQ ID NO: 130 - protein, 442 aa, Homo sapiens
  REGION 1..442: note = Amino acids at position 1 to 442 form Human Immunoglobulin G4 Fc Fragment (homodimer)
  REGION 1..221: note = Amino acids at position 1 to 221 form one monomer
  REGION 222..442: note = Amino acids at position 222 to 442 form one monomer
  DISULFID 3..224: note = Amino acids at position 3 and position 224 form an inter-disulfide bond
  DISULFID 35..95: note = Amino acids at position 35 and position 95 form an intra-chain disulfide bond
  DISULFID 141..199: note = Amino acids at position 141 and position 199 form an intra-chain disulfide bond
  DISULFID 256..316: note = Amino acids at position 256 and position 316 form an intra-chain disulfide bond
  DISULFID 362..420: note = Amino acids at position 362 and position 420 form an intra-chain disulfide bond
PSCPAPEFLGGPSVFLFPPKPKDTLMISRTPEVTCVVVDVSQEDPEVQFNWYVDGVEVHNAKTKPREEQFNSTYRVVSVLTVLHQDWLNGKEYKCKVSNKGLPSSIEKTISKAKGQPREPQVYTLPPSQEEMTKNQVSLTCLVKGFYPSDIAVEWESNGQPENNYKTTPPVLDSDGSFFLYSRLTVDKSRWQEGNVFSCSVMHEALHNHYTQKSLSLSLGKPSCPAPEFLGGPSVFLFPPKPKDTLMISRTPEVTCVVVDVSQEDPEVQFNWYVDGVEVHNAKTKPREEQFNSTYRVVSVLTVLHQDWLNGKEYKCKVSNKGLPSSIEKTISKAKGQPREPQVYTLPPSQEEMTKNQVSLTCLVKGFYPSDIAVEWESNGQPENNYKTTPPVLDSDGSFFLYSRLTVDKSRWQEGNVFSCSVMHEALHNHYTQKSLSLSLGK